European Patent Specification EP 3 656 474 B1, published October 25, 2023. Title: Device for simultaneous and uniform thermal cycling of samples and uses thereof. Applicant: Curiosity Diagnostics Sp. z o.o. The sequence listing filed with the application follows.

SEQUENCE LISTING (4 sequences)

SEQ ID NO: 1 - DNA, 20 bp, Mycobacterium smegmatis
tcttgccctctttctgcttc

SEQ ID NO: 2 - DNA, 22 bp, Mycobacterium smegmatis
cgcaatgattctcgagccgatc

SEQ ID NO: 3 - DNA, 23 bp, Homo sapiens
tctcctctgacttcaacagcgac

SEQ ID NO: 4 - DNA, 22 bp, Homo sapiens
ccctgttgctgtagccaaattc